European Patent Application EP 4 410 305 A1, published August 7, 2024. Title: Anti-cancer vaccine composition comprising HSP90 antigenic peptide and use thereof. Applicant: Aston Sci. The sequence listing filed with the application follows.

SEQUENCE LISTING (2 sequences)

SEQ ID NO: 1 - protein, 15 aa, synthetic construct
LYVRRVFIMDNCEEL

SEQ ID NO: 2 - protein, 15 aa, synthetic construct
  VARIANT 1: note = X is pyroglutamate
XSKILKVIRKNLVKK